European Patent Specification EP 3 436 571 B1, published June 14, 2023. Title: B-cell cultivation method. Applicant: F. Hoffmann-La Roche AG. The sequence listing filed with the application follows.

SEQUENCE LISTING (45 sequences)

SEQ ID NO: 1 - DNA, 32 bp, Artificial Sequence
  rb-V-kappa-HindIIIs primer
gattaagcttatggacaygagggcccccactc

SEQ ID NO: 2 - DNA, 35 bp, Artificial Sequence
  rb-C-kappa-NheIas primer
gatcgctagccctggcaggcgtctcrctctaacag

SEQ ID NO: 3 - DNA, 23 bp, Artificial Sequence
  rb-CH1rev-1 primer
gcagggggccagtgggaagactg

SEQ ID NO: 4 - DNA, 29 bp, Artificial Sequence
  rbVH3-23for3 primer
caccatggagactgggctgcgctggcttc

SEQ ID NO: 5 - DNA, 20 bp, Artificial Sequence
  bcPCR-huCgamma-rev primer
cccccagaggtgctcttgga

SEQ ID NO: 6 - DNA, 20 bp, Artificial Sequence
  bcPCR-FHLC-leader-fw primer
atggacatgagggtccccgc

SEQ ID NO: 7 - DNA, 24 bp, Artificial Sequence
  bcPCR-huCkappa-rev primer
gatttcaactgctcatcagatggc

SEQ ID NO: 8 - DNA, 45 bp, Artificial Sequence
  bcPCR-hu-HC-10600-SLIC-as primer
cagcccagtctccatggtggcaagcttcctctgtgttcagtgctg

SEQ ID NO: 9 - DNA, 26 bp, Artificial Sequence
  bcPCR-hu-HC-10600-SLIC-s  primer
ctccaagagcacctctgggggcacag

SEQ ID NO: 10 - DNA, 24 bp, Artificial Sequence
  bcPCR-hu-LC-10603-SLIC-s  primer
gccatctgatgagcagttgaaatc

SEQ ID NO: 11 - DNA, 38 bp, Artificial Sequence
  bcPCR-hu-LC-10603-SLIC-as  primer
gcggggaccctcatgtccatggtggcaagcttcctctg

SEQ ID NO: 12 - DNA, 48 bp, Artificial Sequence
  SLIC-hu-VHuniversal-for  primer
agcaacagctacaggtgtgcattccgaggtgcagctgktgsagtctgs

SEQ ID NO: 13 - DNA, 45 bp, Artificial Sequence
  SLIC-hu-VH6-for primer
agcaacagctacaggtgtgcattcccaggtrcagctgcagsagtc

SEQ ID NO: 14 - DNA, 24 bp, Artificial Sequence
  hu-CH1gamma-rev primer
gtccaccttggtgttgctgggctt

SEQ ID NO: 15 - DNA, 47 bp, Artificial Sequence
  SLIC-huVk2-for  primer
tagcaacagctacaggtgtgcattccgatgttgtgatgactcagtct

SEQ ID NO: 16 - DNA, 47 bp, Artificial Sequence
  SLIC-huVk3-for  primer
tagcaacagctacaggtgtgcattccgaaattgtgwtgacrcagtct

SEQ ID NO: 17 - DNA, 44 bp, Artificial Sequence
  SLIC-huVk5-for  primer
tagcaacagctacaggtgtgcattccgacatcgtgatgacccag

SEQ ID NO: 18 - DNA, 47 bp, Artificial Sequence
  SLIC-huVk7-for  primer
tagcaacagctacaggtgtgcattccgaaattgtgctgactcagtct

SEQ ID NO: 19 - DNA, 49 bp, Artificial Sequence
  SLIC-huVk8-for  primer
tagcaacagctacaggtgtgcattccgawrttgtgmtgackcagtctcc

SEQ ID NO: 20 - DNA, 47 bp, Artificial Sequence
  SLIC-huVk1long-for  primer
tagcaacagctacaggtgtgcattccgacatccrgwtgacccagtct

SEQ ID NO: 21 - DNA, 47 bp, Artificial Sequence
  SLIC-huVk2longw-for  primer
tagcaacagctacaggtgtgcattccgatrttgtgatgacycagwct

SEQ ID NO: 22 - DNA, 22 bp, Artificial Sequence
  huCk-rev primer
acactctcccctgttgaagctc

SEQ ID NO: 23 - DNA, 44 bp, Artificial Sequence
  SLIC-huVl1-for  primer
tagcaacagctacaggtgtgcattcccagtctgtgytgackcag

SEQ ID NO: 24 - DNA, 44 bp, Artificial Sequence
  SLIC-huVl2-for  primer
tagcaacagctacaggtgtgcattcccagtctgccctgactcag

SEQ ID NO: 25 - DNA, 44 bp, Artificial Sequence
  SLIC-huVl3-for  primer
tagcaacagctacaggtgtgcattcctcctatgagctgaywcag

SEQ ID NO: 26 - DNA, 44 bp, Artificial Sequence
  SLIC-huVl4-for  primer
tagcaacagctacaggtgtgcattcccagcytgtgctgactcaa

SEQ ID NO: 27 - DNA, 44 bp, Artificial Sequence
  SLIC-huVl5-for  primer
tagcaacagctacaggtgtgcattcccagsctgtgctgactcag

SEQ ID NO: 28 - DNA, 44 bp, Artificial Sequence
  SLIC-huVl6-for  primer
tagcaacagctacaggtgtgcattccaattttatgctgactcag

SEQ ID NO: 29 - DNA, 44 bp, Artificial Sequence
  SLIC-huVl7-for  primer
tagcaacagctacaggtgtgcattcccagrctgtggtgactcag

SEQ ID NO: 30 - DNA, 44 bp, Artificial Sequence
  SLIC-huVl8-for  primer
tagcaacagctacaggtgtgcattcccagactgtggtgacccag

SEQ ID NO: 31 - DNA, 44 bp, Artificial Sequence
  SLIC-huVl9-for  primer
tagcaacagctacaggtgtgcattcccwgcctgtgctgactcag

SEQ ID NO: 32 - DNA, 44 bp, Artificial Sequence
  SLIC-huVlambda10-for  primer
tagcaacagctacaggtgtgcattcccaggcagggctgactcag

SEQ ID NO: 33 - DNA, 19 bp, Artificial Sequence
  huCl-1-rev  primer
tctccacggtgctcccttc

SEQ ID NO: 34 - DNA, 26 bp, Artificial Sequence
  huIg-PCR-vectorprimer-as
ggaatgcacacctgtagctgttgcta

SEQ ID NO: 35 - DNA, 24 bp, Artificial Sequence
  huIg-PCR-vectorprimer-VH-s
aagcccagcaacaccaaggtggac

SEQ ID NO: 36 - DNA, 26 bp, Artificial Sequence
  huIg-PCR-vectorprimer-as kappa
ggaatgcacacctgtagctgttgcta

SEQ ID NO: 37 - DNA, 22 bp, Artificial Sequence
  huIg-PCR-vectorprimer-VK-s
gagcttcaacaggggagagtgt

SEQ ID NO: 38 - DNA, 26 bp, Artificial Sequence
  huIg-PCR-vectorprimer-as lambda
ggaatgcacacctgtagctgttgcta

SEQ ID NO: 39 - DNA, 19 bp, Artificial Sequence
  huIg-PCR-vectorprimer-VL-s
gaagggagcaccgtggaga

SEQ ID NO: 40 - protein, 4 aa, Homo sapiens
EVQL

SEQ ID NO: 41 - protein, 4 aa, Homo sapiens
QVQL

SEQ ID NO: 42 - protein, 3 aa, Homo sapiens
VSS

SEQ ID NO: 43 - protein, 4 aa, Homo sapiens
DIVM

SEQ ID NO: 44 - protein, 4 aa, Homo sapiens
DIQM

SEQ ID NO: 45 - protein, 5 aa, Homo sapiens
KLEIK